European Patent Application EP 4 209 512 A1, published July 12, 2023. Title: Development of drug therapeutic agent containing adaptor and use thereof. Applicant: BEIJING TIANNUOJIANCHENG PHARMA TECH CO LTD. The sequence listing filed with the application follows.

SEQUENCE LISTING (123 sequences)

SEQ ID NO: 1 - protein, 306 aa, Homo sapiens
QSIKGNHLVKVYDYQEDGSVLLTCDAEAKNITWFKDGKMIGFLTEDKKKWNLGSNAKDPRGMYQCKGSQNKSKPLQVYYRMCQNCIELNAPEAAGGPSVFLFPPKPKDTLMISRTPEVTCVVVDVSHEDPEVKFNWYVDGVEVHNAKTKPREEQYNSTYRVVSVLTVLHQDWLNGKEYKCKVSNKALPASIEKTISKAKGQPREPQVCTLPPSRDELTKNQVSLSCAVKGFYPSDIAVEWESNGQPENNYKTTPPVLDSDGSFFLVSKLTVDKSRWQQGNVFSCSVMHEALHNHYTQKSLSLSPGK

SEQ ID NO: 2 - protein, 339 aa, Homo sapiens
QDGNEEMGGITQTPYKVSISGTTVILTCPQYPGSEILWQHNDKNIGGDEDDKNIGSDEDHLSLKEFSELEQSGYYVCYPRGSKPEDANFYLYLRARVCENCMEMDAPEAAGGPSVFLFPPKPKDTLMISRTPEVTCVVVDVSHEDPEVKFNWYVDGVEVHNAKTKPREEQYNSTYRVVSVLTVLHQDWLNGKEYKCKVSNKALPASIEKTISKAKGQPREPQVYTLPPCRDELTKNQVSLWCLVKGFYPSDIAVEWESNGQPENNYKTTPPVLDSDGSFFLYSKLTVDKSRWQQGNVFSCSVMHEALHNHYTQKSLSLSPGKGSGLNDIFEAQKIEWHE

SEQ ID NO: 3 - protein, 305 aa, Homo sapiens
QSFEENRKLNVYNQEDGSVLLTCHVKNTNITWFKEGKMIDILTAHKNKWNLGSNTKDPRGVYQCKGSKDKSKTLQVYYRMCQNCIELNAPEAAGGPSVFLFPPKPKDTLMISRTPEVTCVVVDVSHEDPEVKFNWYVDGVEVHNAKTKPREEQYNSTYRVVSVLTVLHQDWLNGKEYKCKVSNKALPASIEKTISKAKGQPREPQVCTLPPSRDELTKNQVSLSCAVKGFYPSDIAVEWESNGQPENNYKTTPPVLDSDGSFFLVSKLTVDKSRWQQGNVFSCSVMHEALHNHYTQKSLSLSPGK

SEQ ID NO: 4 - protein, 330 aa, Homo sapiens
QDGNEEMGSITQTPYQVSISGTTVILTCSQHLGSEAQWQHNGKNKEDSGDRLFLPEFSEMEQSGYYVCYPRGSNPEDASHHLYLKARVCENCMEMDAPEAAGGPSVFLFPPKPKDTLMISRTPEVTCVVVDVSHEDPEVKFNWYVDGVEVHNAKTKPREEQYNSTYRVVSVLTVLHQDWLNGKEYKCKVSNKALPASIEKTISKAKGQPREPQVYTLPPCRDELTKNQVSLWCLVKGFYPSDIAVEWESNGQPENNYKTTPPVLDSDGSFFLYSKLTVDKSRWQQGNVFSCSVMHEALHNHYTQKSLSLSPGKGSGLNDIFEAQKIEWHE

SEQ ID NO: 5 - protein, 109 aa, Homo sapiens
QAVVTQEPSLTVSPGGTVTLTCRSSTGAVTTSNYANWVQQKPGQAPRGLIGGTNKRAPWTPARFSGSLLGGKAALTLSGAQPEDEAEYYCALWYSNLWVFGGGTKLTVL

SEQ ID NO: 6 - DNA, 327 bp, Homo sapiens
caggctgtggtcacacaagagcctagcctgacagtgtctcctggcggcacagtgaccctgacctgtagatcttctacaggcgccgtgaccaccagcaactacgctaattgggtgcagcagaagcccggccaggctcctagaggactgatcggcggaacaaacaagagagccccttggacacccgccagattctctggatctctgctcggcggaaaggccgctctgacactttctggtgctcagcctgaggacgaggccgagtactattgtgccctgtggtacagcaacctgtgggtgttcggcggaggcaccaaactgacagttctg

SEQ ID NO: 7 - protein, 14 aa, Homo sapiens
RSSTGAVTTSNYAN

SEQ ID NO: 8 - protein, 8 aa, Homo sapiens
GGTNKRAP

SEQ ID NO: 9 - protein, 9 aa, Homo sapiens
ALWYSNLWV

SEQ ID NO: 10 - protein, 109 aa, Homo sapiens
QAVVTQEPSLTVSPGGTVTLTCRSSTGAVTTSNYANWVQEKPGQAPRGLIGGTNKRAPWTPARFSGSLLGGKAALTLSGAQPEDEAEYYCALWYSNLWVFGGGTKLTVL

SEQ ID NO: 11 - DNA, 327 bp, Homo sapiens
caggctgtggtcacacaagagcctagcctgacagtgtctcctggcggcacagtgaccctgacctgtagatcttctacaggcgccgtgaccaccagcaactacgctaattgggtgcaggagaagcccggccaggctcctagaggactgatcggcggaacaaacaagagagccccttggacacccgccagattctctggatctctgctcggcggaaaggccgctctgacactttctggtgctcagcctgaggacgaggccgagtactattgtgccctgtggtacagcaacctgtgggtgttcggcggaggcaccaaactgacagttctg

SEQ ID NO: 12 - protein, 109 aa, Homo sapiens
EAVVTQEPSLTVSPGGTVTLTCESSDGAVTTSNYANWVQEKPGQAPRGLIGGTNKEAPWTPARFSGSLLGGKAALTLSGAQPEDEAEYYCALWYSNLWVFGGGTKLTVL

SEQ ID NO: 13 - DNA, 327 bp, Homo sapiens
gaggctgtggtcacacaagagcctagcctgacagtgtctcctggcggcacagtgaccctgacctgtgagtcttctgacggcgccgtgaccaccagcaactacgctaattgggtgcaggagaagcccggccaggctcctagaggactgatcggcggaacaaacaaggaggccccttggacacccgccagattctctggatctctgctcggcggaaaggccgctctgacactttctggtgctcagcctgaggacgaggccgagtactattgtgccctgtggtacagcaacctgtgggtgttcggcggaggcaccaaactgacagttctg

SEQ ID NO: 14 - protein, 14 aa, Homo sapiens
ESSDGAVTTSNYAN

SEQ ID NO: 15 - protein, 8 aa, Homo sapiens
GGTNKEAP

SEQ ID NO: 16 - protein, 109 aa, Homo sapiens
QAVVTQEPSLTVSPGGTVTLTCESSDGAVTTSNYANWVQEKPGQAPRGLIGGTNKEAPWTPARFSGSLLGGKAALTLSGAQPEDEAEYYCALWYSNLWVFGGGTKLTVL

SEQ ID NO: 17 - DNA, 327 bp, Homo sapiens
caggctgtggtcacacaagagcctagcctgacagtgtctcctggcggcacagtgaccctgacctgtgagtcttctgacggcgccgtgaccaccagcaactacgctaattgggtgcaggagaagcccggccaggctcctagaggactgatcggcggaacaaacaaggaggccccttggacacccgccagattctctggatctctgctcggcggaaaggccgctctgacactttctggtgctcagcctgaggacgaggccgagtactattgtgccctgtggtacagcaacctgtgggtgttcggcggaggcaccaaactgacagttctg

SEQ ID NO: 18 - protein, 109 aa, Homo sapiens
QAVVTQEPSLTVSPGGTVTLTCRSSTGAVTTSNYANWVQEKPGQAPRGLIGGTNKRAPWTPARFSGSLLGGKAALTITGAQAEDEAEYYCVLWYSNLWVFGGGTKLTVL

SEQ ID NO: 19 - DNA, 327 bp, Homo sapiens
caggctgtggtcacacaagagcctagcctgacagtgtctcctggcggcacagtgaccctgacctgtagatcttctacaggcgccgtgaccaccagcaactacgctaattgggtgcaggagaagcccggccaggctcctagaggactgatcggcggaacaaacaagagagccccttggacacccgccagattctctggatctctgctcggcggaaaggccgctctgacaatcactggtgctcaggctgaggacgaggccgagtactattgtgtgctgtggtacagcaacctgtgggtgttcggcggaggcaccaaactgacagttctg

SEQ ID NO: 20 - protein, 8 aa, Homo sapiens
YGTNKRAP

SEQ ID NO: 21 - protein, 9 aa, Homo sapiens
VLWYSNLWV

SEQ ID NO: 22 - protein, 109 aa, Homo sapiens
QAVVTQEPSLTVSPGGTVTLTCRSSTGAVTTSNYANWFQEKPGQAPRGLIYGTNKRAPWTPARFSGSLLGGKAALTLSGAQAEDEAEYYCVLWYSNLWVFGGGTKLTVL

SEQ ID NO: 23 - DNA, 327 bp, Homo sapiens
caggctgtggtcacacaagagcctagcctgacagtgtctcctggcggcacagtgaccctgacctgtagatcttctacaggcgccgtgaccaccagcaactacgctaattggttccaggagaagcccggccaggctcctagaggactgatctacggaacaaacaagagagccccttggacacccgccagattctctggatctctgctcggcggaaaggccgctctgacactttctggtgctcaggctgaggacgaggccgagtactattgtgtcctgtggtacagcaacctgtgggtgttcggcggaggcaccaaactgacagttctg

SEQ ID NO: 24 - protein, 125 aa, Homo sapiens
EVQLVESGGGLVQPGGSLRLSCAASGFTFNTYAMNWVRQAPGKGLEWVSRIRSKYNNYATYYADSVKDRFTISRDDSKNTLYLQMNSLKTEDTAVYYCVRHGNFGNSYVSWFAYWGQGTLVTVSS

SEQ ID NO: 25 - DNA, 375 bp, Homo sapiens
gaggtgcagctggttgaatctggcggaggactggttcagcctggcggatctctgagactgtcttgtgccgccagcggcttcaccttcaacacctacgctatgaactgggtccgacaggcccctggcaaaggactggaatgggtgtccagaatcaggtccaagtacaacaactacgccacctactacgccgacagcgtgaaggacagattcaccatcagcagggacgacagcaagaacaccctgtacctgcagatgaacagcctgagagccgaggacaccgccgtgtactactgtgtcagacacggcaacttcggcaacagctatgtgtcttggtttgcctactggggccagggcacactggtcacagttagctct

SEQ ID NO: 26 - protein, 6 aa, Homo sapiens
NTYAMN

SEQ ID NO: 27 - protein, 18 aa, Homo sapiens
IRSKYNNYATYYADSVKD

SEQ ID NO: 28 - protein, 14 aa, Homo sapiens
HGNFGNSYVSWFAY

SEQ ID NO: 29 - protein, 125 aa, Homo sapiens
EVQLVESGGGLVQPGGSLRLSCAASGFTFSTYAMNWVRKAPGKGLEWVSRIRSKYNNYATYYADSVKDRFTISRDDSKNTLYLQMNSLRAEDTAVYYCVRHGNFGNSYVSWFAYWGQGTLVTVSS

SEQ ID NO: 30 - DNA, 375 bp, Homo sapiens
gaggtgcagctggttgaatctggcggaggactggttcagcctggcggatctctgagactgtcttgtgccgccagcggcttcaccttctccacctacgctatgaactgggtccgaaaggcccctggcaaaggactggaatgggtgtccagaatcaggtccaagtacaacaactacgccacctactacgccgacagcgtgaaggacagattcaccatcagcagggacgacagcaagaacaccctgtacctgcagatgaacagcctgagagccgaggacaccgccgtgtactactgtgtcagacacggcaacttcggcaacagctatgtgtcttggtttgcctactggggccagggcacactggtcacagttagctct

SEQ ID NO: 31 - protein, 6 aa, Homo sapiens
STYAMN

SEQ ID NO: 32 - protein, 125 aa, Homo sapiens
EVQLVESGGGLVQPGGSLRLSCAASGFTFSTYAMNWVRKAPGKGLEWVSRIRSKYNNYATYYADSVKDRFTISRDDSKNTLYLQMNSLRAEDTAVYYCVRHGNFGESYVSWFAYWGQGTLVTVSS

SEQ ID NO: 33 - DNA, 375 bp, Homo sapiens
gaggtgcagctggttgaatctggcggaggactggttcagcctggcggatctctgagactgtcttgtgccgccagcggcttcaccttctccacctacgctatgaactgggtccgaaaggcccctggcaaaggactggaatgggtgtccagaatcaggtccaagtacaacaactacgccacctactacgccgacagcgtgaaggacagattcaccatcagcagggacgacagcaagaacaccctgtacctgcagatgaacagcctgagagccgaggacaccgccgtgtactactgtgtcagacacggcaacttcggcgagagctatgtgtcttggtttgcctactggggccagggcacactggtcacagttagctct

SEQ ID NO: 34 - protein, 14 aa, Homo sapiens
HGNFGESYVSWFAY

SEQ ID NO: 35 - protein, 125 aa, Homo sapiens
EVQLVESGGGLVQPGGSLRLSCAASGFTFSTYAMNWVRKAPGKGLEWVSRIRSKYNNYATYYADSVKDRFTISRDDSKNTLYLQMNSLRAEDTAVYYCVRHGNFGQSYVSWFAYWGQGTLVTVSS

SEQ ID NO: 36 - DNA, 375 bp, Homo sapiens
gaggtgcagctggttgaatctggcggaggactggttcagcctggcggatctctgagactgtcttgtgccgccagcggcttcaccttctccacctacgctatgaactgggtccgaaaggcccctggcaaaggactggaatgggtgtccagaatcaggtccaagtacaacaactacgccacctactacgccgacagcgtgaaggacagattcaccatcagcagggacgacagcaagaacaccctgtacctgcagatgaacagcctgagagccgaggacaccgccgtgtactactgtgtcagacacggcaacttcggccagagctatgtgtcttggtttgcctactggggccagggcacactggtcacagttagctct

SEQ ID NO: 37 - protein, 14 aa, Homo sapiens
HGNFGQSYVSWFAY

SEQ ID NO: 38 - protein, 125 aa, Homo sapiens
EVQLVESGGGLVQPGGSLRLSCAASGFTFSTYAMNWVRKAPGKGLEWVSRIRSKYNNYATYYADSVKDRFTISRDDSKNTLYLQMNSLRAEDTAVYYCVRHGNFGDSYVSWFAYWGQGTLVTVSS

SEQ ID NO: 39 - DNA, 375 bp, Homo sapiens
gaggtgcagctggttgaatctggcggaggactggttcagcctggcggatctctgagactgtcttgtgccgccagcggcttcaccttctccacctacgctatgaactgggtccgaaaggcccctggcaaaggactggaatgggtgtccagaatcaggtccaagtacaacaactacgccacctactacgccgacagcgtgaaggacagattcaccatcagcagggacgacagcaagaacaccctgtacctgcagatgaacagcctgagagccgaggacaccgccgtgtactactgtgtcagacacggcaacttcggcgacagctatgtgtcttggtttgcctactggggccagggcacactggtcacagttagctct

SEQ ID NO: 40 - protein, 14 aa, Homo sapiens
HGNFGDSYVSWFAY

SEQ ID NO: 41 - protein, 125 aa, Homo sapiens
EVQLVESGGGLVQPGGSLRLSCAASGFTFSTYAMNWVRKAPGKGLEWVSRIRSKYNNYATYYADSVKDRFTISRDDSKNTLYLQMNSLRAEDTAVYYCVRHGNFGTSYVSWFAYWGQGTLVTVSS

SEQ ID NO: 42 - DNA, 375 bp, Homo sapiens
gaggtgcagctggttgaatctggcggaggactggttcagcctggcggatctctgagactgtcttgtgccgccagcggcttcaccttctccacctacgctatgaactgggtccgaaaggcccctggcaaaggactggaatgggtgtccagaatcaggtccaagtacaacaactacgccacctactacgccgacagcgtgaaggacagattcaccatcagcagggacgacagcaagaacaccctgtacctgcagatgaacagcctgagagccgaggacaccgccgtgtactactgtgtcagacacggcaacttcggcaccagctatgtgtcttggtttgcctactggggccagggcacactggtcacagttagctct

SEQ ID NO: 43 - protein, 14 aa, Homo sapiens
HGNFGTSYVSWFAY

SEQ ID NO: 44 - protein, 125 aa, Homo sapiens
EVQLVESGGGLVQPGGSLRLSCAASGFTFSDYAMNWVRKAPGKGLEWVSRIRSKYNNYATYYADSVEDRFTISRDDSKNTLYLQMNSLRAEDTAVYYCVRHGNFGNSYVSWFAYWGQGTLVTVSS

SEQ ID NO: 45 - DNA, 375 bp, Homo sapiens
gaggtgcagctggttgaatctggcggaggactggttcagcctggcggatctctgagactgtcttgtgccgccagcggcttcaccttctccgactacgctatgaactgggtccgaaaggcccctggcaaaggactggaatgggtgtccagaatcaggtccaagtacaacaactacgccacctactacgccgacagcgtggaggacagattcaccatcagcagggacgacagcaagaacaccctgtacctgcagatgaacagcctgagagccgaggacaccgccgtgtactactgtgtcagacacggcaacttcggcaacagctatgtgtcttggtttgcctactggggccagggcacactggtcacagttagctct

SEQ ID NO: 46 - protein, 6 aa, Homo sapiens
SDYAMN

SEQ ID NO: 47 - protein, 18 aa, Homo sapiens
IRSKYNNYATYYADSVED

SEQ ID NO: 48 - protein, 125 aa, Homo sapiens
EVQLVESGGGLVQPGGSLRLSCAASGFTFNTYAMNWVRKAPGKGLEWVGRIRSKYNNYATYYADSVKDRFTISRDDSKNSLYLQMNSLKTEDTAVYYCARHGNFGNSYVSWFAYWGQGTLVTVSS

SEQ ID NO: 49 - DNA, 375 bp, Homo sapiens
gaggtgcagctggttgaatctggcggaggactggttcagcctggcggatctctgagactgtcttgtgccgccagcggcttcaccttcaacacctacgctatgaactgggtccgaaaggcccctggcaaaggactggaatgggtgggaagaatcaggtccaagtacaacaactacgccacctactacgccgacagcgtgaaggacagattcaccatcagcagggacgacagcaagaacagcctgtacctgcagatgaacagcctgaaaaccgaggacaccgccgtgtactactgtgccagacacggcaacttcggcaacagctatgtgtcttggtttgcctactggggccagggcacactggtcacagttagctct

SEQ ID NO: 50 - protein, 125 aa, Homo sapiens
EVQLVESGGGLVQPGGSLRLSCAASGFTFNTYAMNWVRKAPGKGLEWVGRIRSKYNNYATYYADSVKDRFTISRDDSKNSLYLQMNSLKTEDTAVYYCVRHGNFGNSYVSWFAYWGQGTLVTVSS

SEQ ID NO: 51 - DNA, 375 bp, Homo sapiens
gaggtgcagctggttgaatctggcggaggactggttcagcctggcggatctctgagactgtcttgtgccgccagcggcttcaccttcaacacctacgctatgaactgggtccgaaaggcccctggcaaaggactggaatgggtgggaagaatcaggtccaagtacaacaactacgccacctactacgccgacagcgtgaaggacagattcaccatcagcagggacgacagcaagaacagcctgtacctgcagatgaacagcctgaaaaccgaggacaccgccgtgtactactgtgtcagacacggcaacttcggcaacagctatgtgtcttggtttgcctactggggccagggcacactggtcacagttagctct

SEQ ID NO: 52 - protein, 125 aa, Homo sapiens
EVQLVESGGGLVQPGGSLRLSCAASGFTFNTYAMNWVRKAPGKGLEWVARIRSKYNNYATYYADSVKDRFTISRDDSKNSLYLQMNSLKTEDTAVYYCVRHGNFGNSYVSWFAYWGQGTLVTVSS

SEQ ID NO: 53 - DNA, 375 bp, Homo sapiens
gaggtgcagctggttgaatctggcggaggactggttcagcctggcggatctctgagactgtcttgtgccgccagcggcttcaccttcaacacctacgctatgaactgggtccgaaaggcccctggcaaaggactggaatgggtggccagaatcaggtccaagtacaacaactacgccacctactacgccgacagcgtgaaggacagattcaccatcagcagggacgacagcaagaacagcctgtacctgcagatgaacagcctgaaaaccgaggacaccgccgtgtactactgtgtcagacacggcaacttcggcaacagctatgtgtcttggtttgcctactggggccagggcacactggtcacagttagctct

SEQ ID NO: 54 - protein, 106 aa, Homo sapiens
EIVLTQSPGTLSLSPGERATLSCRASSSVSYIHWFQQKPGQAPRPLIYATSNLASGIPDRFSGSGSGTDYTLTISRLEPEDFAVYYCQQWTSNPPTFGQGTKLEIK

SEQ ID NO: 55 - DNA, 318 bp, Homo sapiens
gagatcgtgctgacacagagccctggcacactgtcactgtctccaggcgagagagccacactgagctgtagagccagcagcagcgtgtcctacatccactggttccagcagaagcctggacaggcccctagacctctgatctacgccacaagcaacctggccagcggcatccctgatagattcagcggctctggcagcggcaccgactacacactgacaatcagcagactggaacccgaggacttcgccgtgtactactgccagcagtggaccagcaatcctcctacattcggccagggcaccaagctggaaatcaag

SEQ ID NO: 56 - protein, 10 aa, Homo sapiens
RASSSVSYIH

SEQ ID NO: 57 - protein, 7 aa, Homo sapiens
ATSNLAS

SEQ ID NO: 58 - protein, 9 aa, Homo sapiens
QQWTSNPPT

SEQ ID NO: 59 - protein, 107 aa, Homo sapiens
EIVLTQSPGTLSLSPGERATLSCRASQSVSSYLAWYQQKPGQAPRLLIYDASNRATGIPDRFSGSGSGTDFTLTISRLEPEDFAVYYCQQRSNWPITFGQGTKLEIK

SEQ ID NO: 60 - DNA, 321 bp, Homo sapiens
gagatcgtgctgacacagagccctggcacactgtcactgtctccaggcgagagagccacactgagctgtagagccagccagagcgtgtcctcttacctggcctggtatcagcagaagcctggacaggctcccagactgctgatctacgacgccagcaacagagccacaggcatccccgatagattcagcggctctggctctggcaccgacttcaccctgacaatcagcagactggaacccgaggacttcgccgtgtactactgccagcagagaagcaactggcccatcacattcggccagggcaccaagctggaaatcaag

SEQ ID NO: 61 - protein, 11 aa, Homo sapiens
RASQSVSSYLA

SEQ ID NO: 62 - protein, 7 aa, Homo sapiens
DASNRAT

SEQ ID NO: 63 - protein, 9 aa, Homo sapiens
QQRSNWPIT

SEQ ID NO: 64 - protein, 121 aa, Homo sapiens
QVQLVQSGAEVKKPGSSVKVSCKASGYTFTSYNMHWVRQAPGQGLEWMGAIYPGNGDTSYNQKFQGRVTLTADKSSSTAYMELSSLRSEDTAVYYCARSTYYGGDWYFNVWGQGTLVTVSS

SEQ ID NO: 65 - DNA, 363 bp, Homo sapiens
caggttcagctggttcagtctggcgccgaagtgaagaaacctggcagcagcgtgaaggtgtcctgcaaggctagcggctacacattcaccagctacaacatgcactgggtccgacaggcccctggacagggacttgaatggatgggcgctatctaccctggcaacggcgacacctcctacaaccagaaattccagggcagagtgaccctgaccgccgacaagtctagcagcaccgcctacatggaactgagcagcctgagaagcgaggacaccgccgtgtactactgtgccagaagcacctactacggcggcgactggtacttcaacgtgtggggacagggaaccctggtcaccgtttcttct

SEQ ID NO: 66 - protein, 5 aa, Homo sapiens
SYNMH

SEQ ID NO: 67 - protein, 17 aa, Homo sapiens
AIYPGNGDTSYNQKFQG

SEQ ID NO: 68 - protein, 12 aa, Homo sapiens
STYYGGDWYFNV

SEQ ID NO: 69 - protein, 121 aa, Homo sapiens
QVQLVQSGAEVKKPGSSVKVSCKASGYTFTSYNMHWVRQAPGQGLEWMGAIYPGNGDTSYNQKFQGRVTLTADKSSSTAYMELSSLRSEDTAVYYCARSTYYGGDWYFDYWGQGTLVTVSS

SEQ ID NO: 70 - DNA, 363 bp, Homo sapiens
caggttcagctggttcagtctggcgccgaagtgaagaaacctggcagcagcgtgaaggtgtcctgcaaggctagcggctacacattcaccagctacaacatgcactgggtccgacaggcccctggacagggacttgaatggatgggcgctatctaccctggcaacggcgacacctcctacaaccagaaattccagggcagagtgaccctgaccgccgacaagtctagcagcaccgcctacatggaactgagcagcctgagaagcgaggacaccgccgtgtactactgtgccagaagcacctactacggcggcgactggtacttcgactattggggacagggaaccctggtcaccgtttcttct

SEQ ID NO: 71 - protein, 12 aa, Homo sapiens
STYYGGDWYFDY

SEQ ID NO: 72 - protein, 121 aa, Homo sapiens
EVQLVESGGGLVQPGGSLRLSCAASGYTFTSYNMHWVRQAPGQGLEWMGAIYPGNGDTSYNQKFQGRVTLTADKSSSTAYMELSSLRSEDTAVYYCARSTYYGGDWYFNVWGQGTLVTVSS

SEQ ID NO: 73 - DNA, 363 bp, Homo sapiens
gaggtgcagctggttgaatctggcggaggactggttcagcctggcggatctctgagactgtcttgtgccgccagcggctacaccttcaccagctacaatatgcactgggtccgacaggcccctggacagggacttgaatggatgggcgctatctaccctggcaacggcgacacctcctacaaccagaaattccagggcagagtgaccctgaccgccgacaagtctagcagcaccgcctacatggaactgagcagcctgagaagcgaggacaccgccgtgtactactgtgccagaagcacctactacggcggcgactggtacttcaacgtgtggggacagggaaccctggtcaccgtttcttct

SEQ ID NO: 74 - protein, 122 aa, Homo sapiens
EVQLLESGGGLVQPGGSLRLSCAASGFTFNDYAMHWVRQAPGKGLEWVSTISWNSGSIGYADSVKGRFTISRDNAKKTLYLQMNSLRAEDTAVYYCAKDIQYGNYYYGMDVWGQGTLVTVSS

SEQ ID NO: 75 - DNA, 366 bp, Homo sapiens
gaagtgcagctgctggaatctggcggaggactggttcaacctggcggctctctgagactgtcttgtgccgcttctggcttcaccttcaacgactacgccatgcactgggtccgacaggcccctggaaaaggactggaatgggtgtccaccatcagctggaacagcggctctatcggctacgccgattccgtgaagggcagattcaccatctccagagacaacgccaagaaaaccctgtacctgcagatgaacagcctgagagccgaggacaccgccgtgtactactgtgccaaggacatccagtacggcaactactactacggcatggacgtgtggggccagggaacactggttaccgttagctct

SEQ ID NO: 76 - protein, 5 aa, Homo sapiens
DYAMH

SEQ ID NO: 77 - protein, 17 aa, Homo sapiens
TISWNSGSIGYADSVKG

SEQ ID NO: 78 - protein, 13 aa, Homo sapiens
DIQYGNYYYGMDV

SEQ ID NO: 79 - protein, 122 aa, Homo sapiens
EVQLLESGGGLVQPGGSLRLSCAASGFTFNDYAMHWVRQAPGKGLEWVSTISWNSGSIGYADSVKGRFTISRDNSKNTLYLQMNSLRAEDTAVYYCAKDIQYGNYYYGMDVWGQGTLVTVSS

SEQ ID NO: 80 - DNA, 366 bp, Homo sapiens
gaagtgcagctgctggaatctggtggcggactggttcagcctggcggctctctgagactgtcttgtgctgccagcggcttcaccttcaacgactacgctatgcactgggtccgacaggcccctggcaaaggacttgaatgggtgtccaccatcagctggaacagcggctctatcggctacgccgattccgtgaagggcagattcaccatctccagagacaacagcaagaacaccctgtacctgcagatgaacagcctgagagccgaggacaccgccgtgtactactgtgccaaggacatccagtacggcaactactactacggcatggacgtgtggggccagggaacactggttaccgttagctct

SEQ ID NO: 81 - protein, 122 aa, Homo sapiens
EVQLLESGGGVVQPGGSLRLSCAASGFTFNDYAMHWVRQAPGKGLEWVSTISWNSGSIGYADSVKGRFTISRDNSKNTLYLQMNSLRAEDTAVYYCAKDIQYGNYYYGMDVWGQGTLVTVSS

SEQ ID NO: 82 - DNA, 366 bp, Homo sapiens
gaagtgcagctgctggaatctggtggcggagttgttcagcctggcggctctctgagactgtcttgtgctgccagcggcttcaccttcaacgactacgctatgcactgggtccgacaggcccctggcaaaggacttgaatgggtgtccaccatcagctggaacagcggctctatcggctacgccgattccgtgaagggcagattcaccatctccagagacaacagcaagaacaccctgtacctgcagatgaacagcctgagagccgaggacaccgccgtgtactactgtgccaaggacatccagtacggcaactactactacggcatggacgtgtggggccagggaacactggttaccgttagctct

SEQ ID NO: 83 - protein, 122 aa, Homo sapiens
EVQLLESGGGVVQPGGSLRLSCAASGFTFNDYAMHWVRQAPGKGLEWVSTISWNSGSIGYADSVKGRFTISRDNSKNTLYLQMNSLRAEDTAVYYCAKDIQYGNYYYGMDYWGQGTLVTVSS

SEQ ID NO: 84 - DNA, 366 bp, Homo sapiens
gaagtgcagctgctggaatctggtggcggagttgttcagcctggcggctctctgagactgtcttgtgctgccagcggcttcaccttcaacgactacgctatgcactgggtccgacaggcccctggcaaaggacttgaatgggtgtccaccatcagctggaacagcggctctatcggctacgccgattccgtgaagggcagattcaccatctccagagacaacagcaagaacaccctgtacctgcagatgaacagcctgagagccgaggacaccgccgtgtactactgtgccaaggacatccagtacggcaactactactacggcatggactactggggccagggaacactggttaccgttagctct

SEQ ID NO: 85 - protein, 13 aa, Homo sapiens
DIQYGNYYYGMDY

SEQ ID NO: 86 - protein, 448 aa, Homo sapiens
QVQLVQSGAEVKKPGSSVKVSCKASGYTFTSYNMHWVREAPGQGLEWMGAIYPGNGDTSYNQKFQGRVTLTADKSSSTAYMELSSLRSEDTAVYYCARSTYYGGDWYFDYWGQGTLVTVSSASTKGPSVFPLAPCSRSTSESTAALGCLVEDYFPEPVTVSWNSGALTSGVHTFPAVLQSSGLYSLSSVVTVPSSSLGTKTYTCNVDHKPSNTKVDERVESKYGPPCPPCPAPEFEGGPSVFLFPPKPKDTLMISRTPEVTCVVVDVSQEDPEVQFNWYVDGVEVHNAKTKPREEQFASTYRVVSVLTVLHQDWLNGKEYKCKVSNKGLPSSIEKTISKAKGQPREPQVCTLPPSQEEMTKNQVSLSCAVKGFYPSDIAVEWESNGQPENNYKTTPPVLDSDGSFFLVSKLTVDKSRWQEGNVFSCSVMHEALHNHYTQKSLSLSLGK

SEQ ID NO: 87 - DNA, 1344 bp, Homo sapiens
caggttcagctggttcagtctggcgccgaagtgaagaaacctggcagcagcgtgaaggtgtcctgcaaggctagcggctacacattcaccagctacaacatgcactgggtccgagaggcccctggacagggacttgaatggatgggcgctatctaccctggcaacggcgacacctcctacaaccagaaattccagggcagagtgaccctgaccgccgacaagtctagcagcaccgcctacatggaactgagcagcctgagaagcgaggacaccgccgtgtactactgtgccagaagcacctactacggcggcgactggtacttcgactattggggacagggaaccctggtcaccgtttcttctgctagcaccaagggccccagcgtgttccccctggccccttgcagcagaagcaccagcgagagcacagccgccctgggctgcctggtggaggactacttccccgagcccgtgaccgtgtcctggaacagcggcgctctgaccagcggcgtgcataccttccccgccgtgctccagagcagcggactgtactccctgagcagcgtggtgaccgtgccttccagcagcctgggcaccaagacctacacctgcaacgtggaccacaagcccagcaacaccaaggtggacgagagagtggagagcaagtacggccctccctgccccccttgccctgcccccgagttcgaaggcggacctagcgtgttcctgttcccccccaagcccaaggacaccctgatgatcagcagaacccccgaggtgacctgcgtggtggtggacgtgtcccaggaggaccccgaggtccagtttaattggtacgtggacggcgtggaagtgcataacgccaagaccaagcccagagaggagcagttcgccagcacctacagagtggtgtccgtgctgaccgtgctgcaccaggactggctgaacggcaaggaatacaagtgcaaggtctccaacaagggcctgcctagcagcatcgagaagaccatcagcaaggccaagggccagccacgggagccccaggtctgcaccctgccacctagccaagaggagatgaccaagaaccaggtgtccctgagctgtgccgtgaaaggcttctatcccagcgatatcgccgtggagtgggagagcaacggccagcccgagaacaactacaagaccaccccccctgtgctggacagcgacggcagcttcttcctggtttccaagctgaccgtggacaagtccagatggcaggagggcaacgtcttcagctgctccgtgatgcacgaggccctgcacaaccactacacccagaagtccctgagcctgagcctgggcaag

SEQ ID NO: 88 - protein, 213 aa, Homo sapiens
EIVLTQSPGTLSLSPGERATLSCRASSSVSYIHWFQKKPGQAPRPLIYATSNLASGIPDRFSGSGSGTDYTLTISRLEPEDFAVYYCQQWTSNPPTFGQGTKLEIKRTVAAPSVFIFPPSDKKLKSGTASVVCLLNNFYPREAKVQWKVDNALQSGNSQESVTEQDSKDSTYSLSSTLTLSKADYEKHKVYACEVTHQGLSSPVTKSFNRGEC

SEQ ID NO: 89 - DNA, 639 bp, Homo sapiens
gagatcgtgctgacacagagccctggcacactgtcactgtctccaggcgagagagccacactgagctgtagagccagcagcagcgtgtcctacatccactggttccagaagaagcctggacaggcccctagacctctgatctacgccacaagcaacctggccagcggcatccctgatagattcagcggctctggcagcggcaccgactacacactgacaatcagcagactggaacccgaggacttcgccgtgtactactgccagcagtggaccagcaatcctcctacattcggccagggcaccaagctggaaatcaagcgaactgtggctgcaccatctgtcttcatcttcccgccatctgataagaaattgaaatctggaactgcctctgttgtgtgcctgctgaataacttctatcccagagaggccaaagtacagtggaaggtggataacgccctccaatcgggtaactcccaggagagtgtcacagagcaggacagcaaggacagcacctacagcctcagcagcaccctgacgctgagcaaagcagactacgagaaacacaaagtctacgcctgcgaagtcacccatcagggcctgagctcgcccgtcacaaagagcttcaacaggggagagtgt

SEQ ID NO: 90 - protein, 444 aa, Homo sapiens
QAVVTQEPSLTVSPGGTVTLTCRSSTGAVTTSNYANWVQEKPGQAPRGLIGGTNKRAPWTPARFSGSLLGGKAALTITGAQAEDEAEYYCVLWYSNLWVFGGGTKLTVLGQPKAAPSVTLFPPSSEELQANKATLVCLISDFYPGAVTVAWKADSSPVKAGVETTTPSKQSNNKYAASSYLSLTPEQWKSHRSYSCQVTHEGSTVEKTVAPTECSESKYGPPCPPCPAPEFEGGPSVFLFPPKPKDTLMISRTPEVTCVVVDVSQEDPEVQFNWYVDGVEVHNAKTKPREEQFASTYRVVSVLTVLHQDWLNGKEYKCKVSNKGLPSSIEKTISKAKGQPREPQVYTLPPCQEEMTKNQVSLWCLVKGFYPSDIAVEWESNGQPENNYKTTPPVLDSDGSFFLYSKLTVDKSRWQEGNVFSCSVMHEALHNHYTQKSLSLSLGK

SEQ ID NO: 91 - DNA, 1332 bp, Homo sapiens
caggctgtggtcacacaagagcctagcctgacagtgtctcctggcggcacagtgaccctgacctgtagatcttctacaggcgccgtgaccaccagcaactacgctaattgggtgcaggagaagcccggccaggctcctagaggactgatcggcggaacaaacaagagagccccttggacacccgccagattctctggatctctgctcggcggaaaggccgctctgacaatcactggtgctcaggctgaggacgaggccgagtactattgtgtgctgtggtacagcaacctgtgggtgttcggcggaggcaccaaactgacagttctgggtcagcccaaggcggcgccctcggtcactctgttcccgccctcctctgaggagcttcaagccaacaaggccacactggtgtgtctcataagtgacttctatccgggagccgtgacagtggcctggaaggcagatagcagccccgtcaaggcgggagtggagaccaccacaccctccaaacaaagcaacaacaagtacgcggccagcagctacctgagcctgacgcctgagcagtggaagtcccacagaagctacagctgccaggtcacgcatgaagggagcaccgtggagaagacagtggcccctacagaatgttcagagagcaagtacggccctccctgccccccttgccctgcccccgagttcgagggcggacctagcgtgttcctgttcccccccaagcccaaggacaccctgatgatcagcagaacccccgaggtgacctgcgtggtggtggacgtgtcccaggaggaccccgaggtccagtttaattggtacgtggacggcgtggaagtgcataacgccaagaccaagcccagagaggagcagttcgccagcacctacagagtggtgtccgtgctgaccgtgctgcaccaggactggctgaacggcaaggaatacaagtgcaaggtctccaacaagggcctgcctagcagcatcgagaagaccatcagcaaggccaagggccagccacgggagccccaggtctacaccctgccaccttgtcaagaggagatgaccaagaaccaggtgtccctgtggtgtctggtgaaaggcttctatcccagcgatatcgccgtggagtgggagagcaacggccagcccgagaacaactacaagaccaccccccctgtgctggacagcgacggcagcttcttcctgtactccaagctgaccgtggacaagtccagatggcaggagggcaacgtcttcagctgctccgtgatgcacgaggccctgcacaaccactacacccagaagtccctgagcctgagcctgggcaag

SEQ ID NO: 92 - protein, 223 aa, Homo sapiens
EVQLVESGGGLVQPGGSLRLSCAASGFTFNTYAMNWVRKAPGKGLEWVGRIRSKYNNYATYYADSVKDRFTISRDDSKNSLYLQMNSLKTEDTAVYYCVRHGNFGNSYVSWFAYWGQGTLVTVSSASTKGPSVFPLAPCSRSTSESTAALGCLVKDYFPEPVTVSWNSGALTSGVHTFPAVLQSSGLYSLSSVVTVPSSSLGTKTYTCNVDHKPSNTKVDKRV

SEQ ID NO: 93 - DNA, 669 bp, Homo sapiens
gaggtgcagctggttgaatctggcggaggactggttcagcctggcggatctctgagactgtcttgtgccgccagcggcttcaccttcaacacctacgctatgaactgggtccgaaaggcccctggcaaaggactggaatgggtgggaagaatcaggtccaagtacaacaactacgccacctactacgccgacagcgtgaaggacagattcaccatcagcagggacgacagcaagaacagcctgtacctgcagatgaacagcctgaaaaccgaggacaccgccgtgtactactgtgtcagacacggcaacttcggcaacagctatgtgtcttggtttgcctactggggccagggcacactggtcacagttagctctgctagcaccaagggccccagcgtgttccccctggccccttgcagcagaagcaccagcgagagcacagccgccctgggctgcctggtgaaggactacttccccgagcccgtgaccgtgtcctggaacagcggcgctctgaccagcggcgtgcataccttccccgccgtgctccagagcagcggactgtactccctgagcagcgtggtgaccgtgccttccagcagcctgggcaccaagacctacacctgcaacgtggaccacaagcccagcaacaccaaggtggacaagagagtg

SEQ ID NO: 94 - protein, 449 aa, Homo sapiens
EVQLLESGGGLVQPGGSLRLSCAASGFTFNDYAMHWVREAPGKGLEWVSTISWNSGSIGYADSVKGRFTISRDNSKNTLYLQMNSLRAEDTAVYYCAKDIQYGNYYYGMDVWGQGTLVTVSSASTKGPSVFPLAPCSRSTSESTAALGCLVEDYFPEPVTVSWNSGALTSGVHTFPAVLQSSGLYSLSSVVTVPSSSLGTKTYTCNVDHKPSNTKVDERVESKYGPPCPPCPAPEFEGGPSVFLFPPKPKDTLMISRTPEVTCVVVDVSQEDPEVQFNWYVDGVEVHNAKTKPREEQFASTYRVVSVLTVLHQDWLNGKEYKCKVSNKGLPSSIEKTISKAKGQPREPQVCTLPPSQEEMTKNQVSLSCAVKGFYPSDIAVEWESNGQPENNYKTTPPVLDSDGSFFLVSKLTVDKSRWQEGNVFSCSVMHEALHNHYTQKSLSLSLGK

SEQ ID NO: 95 - DNA, 1347 bp, Homo sapiens
gaagtgcagctgctggaatctggtggcggactggttcagcctggcggctctctgagactgtcttgtgctgccagcggcttcaccttcaacgactacgctatgcactgggtccgagaggcccctggcaaaggacttgaatgggtgtccaccatcagctggaacagcggctctatcggctacgccgattccgtgaagggcagattcaccatctccagagacaacagcaagaacaccctgtacctgcagatgaacagcctgagagccgaggacaccgccgtgtactactgtgccaaggacatccagtacggcaactactactacggcatggacgtgtggggccagggaacactggttaccgttagctctgctagcaccaagggccccagcgtgttccccctggccccttgcagcagaagcaccagcgagagcacagccgccctgggctgcctggtggaggactacttccccgagcccgtgaccgtgtcctggaacagcggcgctctgaccagcggcgtgcataccttccccgccgtgctccagagcagcggactgtactccctgagcagcgtggtgaccgtgccttccagcagcctgggcaccaagacctacacctgcaacgtggaccacaagcccagcaacaccaaggtggacgagagagtggagagcaagtacggccctccctgccccccttgccctgcccccgagttcgaaggcggacctagcgtgttcctgttcccccccaagcccaaggacaccctgatgatcagcagaacccccgaggtgacctgcgtggtggtggacgtgtcccaggaggaccccgaggtccagtttaattggtacgtggacggcgtggaagtgcataacgccaagaccaagcccagagaggagcagttcgccagcacctacagagtggtgtccgtgctgaccgtgctgcaccaggactggctgaacggcaaggaatacaagtgcaaggtctccaacaagggcctgcctagcagcatcgagaagaccatcagcaaggccaagggccagccacgggagccccaggtctgcaccctgccacctagccaagaggagatgaccaagaaccaggtgtccctgagctgtgccgtgaaaggcttctatcccagcgatatcgccgtggagtgggagagcaacggccagcccgagaacaactacaagaccaccccccctgtgctggacagcgacggcagcttcttcctggtttccaagctgaccgtggacaagtccagatggcaggagggcaacgtcttcagctgctccgtgatgcacgaggccctgcacaaccactacacccagaagtccctgagcctgagcctgggcaag

SEQ ID NO: 96 - protein, 214 aa, Homo sapiens
EIVLTQSPGTLSLSPGERATLSCRASQSVSSYLAWYQKKPGQAPRLLIYDASNRATGIPDRFSGSGSGTDFTLTISRLEPEDFAVYYCQQRSNWPITFGQGTKLEIKRTVAAPSVFIFPPSDKKLKSGTASVVCLLNNFYPREAKVQWKVDNALQSGNSQESVTEQDSKDSTYSLSSTLTLSKADYEKHKVYACEVTHQGLSSPVTKSFNRGEC

SEQ ID NO: 97 - DNA, 642 bp, Homo sapiens
gagatcgtgctgacacagagccctggcacactgtcactgtctccaggcgagagagccacactgagctgtagagccagccagagcgtgtcctcttacctggcctggtatcagaagaagcctggacaggctcccagactgctgatctacgacgccagcaacagagccacaggcatccccgatagattcagcggctctggctctggcaccgacttcaccctgacaatcagcagactggaacccgaggacttcgccgtgtactactgccagcagagaagcaactggcccatcacattcggccagggcaccaagctggaaatcaagcgaactgtggctgcaccatctgtcttcatcttcccgccatctgataagaaattgaaatctggaactgcctctgttgtgtgcctgctgaataacttctatcccagagaggccaaagtacagtggaaggtggataacgccctccaatcgggtaactcccaggagagtgtcacagagcaggacagcaaggacagcacctacagcctcagcagcaccctgacgctgagcaaagcagactacgagaaacacaaagtctacgcctgcgaagtcacccatcagggcctgagctcgcccgtcacaaagagcttcaacaggggagagtgt

SEQ ID NO: 98 - protein, 449 aa, Homo sapiens
EVQLLESGGGVVQPGGSLRLSCAASGFTFNDYAMHWVREAPGKGLEWVSTISWNSGSIGYADSVKGRFTISRDNSKNTLYLQMNSLRAEDTAVYYCAKDIQYGNYYYGMDYWGQGTLVTVSSASTKGPSVFPLAPCSRSTSESTAALGCLVEDYFPEPVTVSWNSGALTSGVHTFPAVLQSSGLYSLSSVVTVPSSSLGTKTYTCNVDHKPSNTKVDERVESKYGPPCPPCPAPEFEGGPSVFLFPPKPKDTLMISRTPEVTCVVVDVSQEDPEVQFNWYVDGVEVHNAKTKPREEQFASTYRVVSVLTVLHQDWLNGKEYKCKVSNKGLPSSIEKTISKAKGQPREPQVCTLPPSQEEMTKNQVSLSCAVKGFYPSDIAVEWESNGQPENNYKTTPPVLDSDGSFFLVSKLTVDKSRWQEGNVFSCSVMHEALHNHYTQKSLSLSLGK

SEQ ID NO: 99 - DNA, 1347 bp, Homo sapiens
gaagtgcagctgctggaatctggtggcggagttgttcagcctggcggctctctgagactgtcttgtgctgccagcggcttcaccttcaacgactacgctatgcactgggtccgagaggcccctggcaaaggacttgaatgggtgtccaccatcagctggaacagcggctctatcggctacgccgattccgtgaagggcagattcaccatctccagagacaacagcaagaacaccctgtacctgcagatgaacagcctgagagccgaggacaccgccgtgtactactgtgccaaggacatccagtacggcaactactactacggcatggactactggggccagggaacactggttaccgttagctctgctagcaccaagggccccagcgtgttccccctggccccttgcagcagaagcaccagcgagagcacagccgccctgggctgcctggtggaggactacttccccgagcccgtgaccgtgtcctggaacagcggcgctctgaccagcggcgtgcataccttccccgccgtgctccagagcagcggactgtactccctgagcagcgtggtgaccgtgccttccagcagcctgggcaccaagacctacacctgcaacgtggaccacaagcccagcaacaccaaggtggacgagagagtggagagcaagtacggccctccctgccccccttgccctgcccccgagttcgaaggcggacctagcgtgttcctgttcccccccaagcccaaggacaccctgatgatcagcagaacccccgaggtgacctgcgtggtggtggacgtgtcccaggaggaccccgaggtccagtttaattggtacgtggacggcgtggaagtgcataacgccaagaccaagcccagagaggagcagttcgccagcacctacagagtggtgtccgtgctgaccgtgctgcaccaggactggctgaacggcaaggaatacaagtgcaaggtctccaacaagggcctgcctagcagcatcgagaagaccatcagcaaggccaagggccagccacgggagccccaggtctgcaccctgccacctagccaagaggagatgaccaagaaccaggtgtccctgagctgtgccgtgaaaggcttctatcccagcgatatcgccgtggagtgggagagcaacggccagcccgagaacaactacaagaccaccccccctgtgctggacagcgacggcagcttcttcctggtttccaagctgaccgtggacaagtccagatggcaggagggcaacgtcttcagctgctccgtgatgcacgaggccctgcacaaccactacacccagaagtccctgagcctgagcctgggcaag

SEQ ID NO: 100 - protein, 214 aa, Homo sapiens; identical to SEQ ID NO: 96

SEQ ID NO: 101 - DNA, 642 bp, Homo sapiens; identical to SEQ ID NO: 97

SEQ ID NO: 102 - protein, 214 aa, Homo sapiens
EIVLTQSPGTLSLSPGERATLSCRASQSVSSYLAWYQQKPGQAPRLLIYDASNRATGIPDRFSGSGSGTDFTLTISRLEPEDFAVYYCQQRSNWPITFGQGTKLEIKRTVAAPSVFIFPPSDEQLKSGTASVVCLLNNFYPREAKVQWKVDNALQSGNSQESVTEQDSKDSTYSLSSTLTLSKADYEKHKVYACEVTHQGLSSPVTKSFNRGEC

SEQ ID NO: 103 - DNA, 642 bp, Homo sapiens
gagatcgtgctgacacagagccctggcacactgtcactgtctccaggcgagagagccacactgagctgtagagccagccagagcgtgtcctcttacctggcctggtatcagcagaagcctggacaggctcccagactgctgatctacgacgccagcaacagagccacaggcatccccgatagattcagcggctctggctctggcaccgacttcaccctgacaatcagcagactggaacccgaggacttcgccgtgtactactgccagcagagaagcaactggcccatcacattcggccagggcaccaagctggaaatcaagcgaactgtggctgcaccatctgtcttcatcttcccgccatctgatgagcagttgaaatctggaactgcctctgttgtgtgcctgctgaataacttctatcccagagaggccaaagtacagtggaaggtggataacgccctccaatcgggtaactcccaggagagtgtcacagagcaggacagcaaggacagcacctacagcctcagcagcaccctgacgctgagcaaagcagactacgagaaacacaaagtctacgcctgcgaagtcacccatcagggcctgagctcgcccgtcacaaagagcttcaacaggggagagtgt

SEQ ID NO: 104 - protein, 449 aa, Homo sapiens
EVQLLESGGGVVQPGGSLRLSCAASGFTFNDYAMHWVRQAPGKGLEWVSTISWNSGSIGYADSVKGRFTISRDNSKNTLYLQMNSLRAEDTAVYYCAKDIQYGNYYYGMDYWGQGTLVTVSSASTKGPSVFPLAPCSRSTSESTAALGCLVKDYFPEPVTVSWNSGALTSGVHTFPAVLQSSGLYSLSSVVTVPSSSLGTKTYTCNVDHKPSNTKVDKRVESKYGPPCPPCPAPEFEGGPSVFLFPPKPKDTLMISRTPEVTCVVVDVSQEDPEVQFNWYVDGVEVHNAKTKPREEQFNSTYRVVSVLTVLHQDWLNGKEYKCKVSNKGLASSIEKTISKAKGQPREPQVCTLPPSQEEMTKNQVSLSCAVKGFYPSDIAVEWESNGQPENNYKTTPPVLDSDGSFFLVSKLTVDKSRWQEGNVFSCSVMHEALHNHYTQKSLSLSLGK

SEQ ID NO: 105 - DNA, 1347 bp, Homo sapiens
gaagtgcagctgctggaatctggtggcggagttgttcagcctggcggctctctgagactgtcttgtgctgccagcggcttcaccttcaacgactacgctatgcactgggtccgacaggcccctggcaaaggacttgaatgggtgtccaccatcagctggaacagcggctctatcggctacgccgattccgtgaagggcagattcaccatctccagagacaacagcaagaacaccctgtacctgcagatgaacagcctgagagccgaggacaccgccgtgtactactgtgccaaggacatccagtacggcaactactactacggcatggactactggggccagggaacactggttaccgttagctctgctagcaccaagggccccagcgtgttccccctggccccttgcagcagaagcaccagcgagagcacagccgccctgggctgcctggtgaaggactacttccccgagcccgtgaccgtgtcctggaacagcggcgctctgaccagcggcgtgcataccttccccgccgtgctccagagcagcggactgtactccctgagcagcgtggtgaccgtgccttccagcagcctgggcaccaagacctacacctgcaacgtggaccacaagcccagcaacaccaaggtggacaagagagtggagagcaagtacggccctccctgccccccttgccctgcccccgagttcgagggcggacctagcgtgttcctgttcccccccaagcccaaggacaccctgatgatcagcagaacccccgaggtgacctgcgtggtggtggacgtgtcccaggaggaccccgaggtccagtttaattggtacgtggacggcgtggaagtgcataacgccaagaccaagcccagagaggagcagttcaacagcacctacagagtggtgtccgtgctgaccgtgctgcaccaggactggctgaacggcaaggaatacaagtgcaaggtctccaacaagggcctggccagcagcatcgagaagaccatcagcaaggccaagggccagccacgggagccccaggtctgcaccctgccacctagccaagaggagatgaccaagaaccaggtgtccctgagctgtgccgtgaaaggcttctatcccagcgatatcgccgtggagtgggagagcaacggccagcccgagaacaactacaagaccaccccccctgtgctggacagcgacggcagcttcttcctggtttccaagctgaccgtggacaagtccagatggcaggagggcaacgtcttcagctgctccgtgatgcacgaggccctgcacaaccactacacccagaagtccctgagcctgagcctgggcaag

SEQ ID NO: 106 - protein, 215 aa, Homo sapiens
QAVVTQEPSLTVSPGGTVTLTCRSSTGAVTTSNYANWVQQKPGQAPRGLIGGTNKRAPWTPARFSGSLLGGKAALTITGAQAEDEAEYYCVLWYSNLWVFGGGTKLTVLGQPKAAPSVTLFPPSSEELQANKATLVCLISDFYPGAVTVAWKADSSPVKAGVETTTPSKQSNNKYAASSYLSLTPEQWKSHRSYSCQVTHEGSTVEKTVAPTECS

SEQ ID NO: 107 - DNA, 645 bp, Homo sapiens
caggctgtggtcacacaagagcctagcctgacagtgtctcctggcggcacagtgaccctgacctgtagatcttctacaggcgccgtgaccaccagcaactacgctaattgggtgcagcagaagcccggccaggctcctagaggactgatcggcggaacaaacaagagagccccttggacacccgccagattctctggatctctgctcggcggaaaggccgctctgacaatcactggtgctcaggctgaggacgaggccgagtactattgtgtgctgtggtacagcaacctgtgggtgttcggcggaggcaccaaactgacagttctgggtcagcccaaggcggcgccctcggtcactctgttcccgccctcctctgaggagcttcaagccaacaaggccacactggtgtgtctcataagtgacttctatccgggagccgtgacagtggcctggaaggcagatagcagccccgtcaaggcgggagtggagaccaccacaccctccaaacaaagcaacaacaagtacgcggccagcagctacctgagcctgacgcctgagcagtggaagtcccacagaagctacagctgccaggtcacgcatgaagggagcaccgtggagaagacagtggcccctacagaatgttca

SEQ ID NO: 108 - protein, 452 aa, Homo sapiens
EVQLVESGGGLVQPGGSLRLSCAASGFTFNTYAMNWVRQAPGKGLEWVGRIRSKYNNYATYYADSVKDRFTISRDDSKNSLYLQMNSLKTEDTAVYYCVRHGNFGNSYVSWFAYWGQGTLVTVSSASTKGPSVFPLAPCSRSTSESTAALGCLVKDYFPEPVTVSWNSGALTSGVHTFPAVLQSSGLYSLSSVVTVPSSSLGTKTYTCNVDHKPSNTKVDKRVESKYGPPCPPCPAPEFEGGPSVFLFPPKPKDTLMISRTPEVTCVVVDVSQEDPEVQFNWYVDGVEVHNAKTKPREEQFNSTYRVVSVLTVLHQDWLNGKEYKCKVSNKGLASSIEKTISKAKGQPREPQVYTLPPCQEEMTKNQVSLWCLVKGFYPSDIAVEWESNGQPENNYKTTPPVLDSDGSFFLYSKLTVDKSRWQEGNVFSCSVMHEALHNHYTQKSLSLSLGK

SEQ ID NO: 109 - DNA, 1356 bp, Homo sapiens
gaggtgcagctggttgaatctggcggaggactggttcagcctggcggatctctgagactgtcttgtgccgccagcggcttcaccttcaacacctacgctatgaactgggtccgacaggcccctggcaaaggactggaatgggtgggaagaatcaggtccaagtacaacaactacgccacctactacgccgacagcgtgaaggacagattcaccatcagcagggacgacagcaagaacagcctgtacctgcagatgaacagcctgaaaaccgaggacaccgccgtgtactactgtgtcagacacggcaacttcggcaacagctatgtgtcttggtttgcctactggggccagggcacactggtcacagttagctctgctagcaccaagggccccagcgtgttccccctggccccttgcagcagaagcaccagcgagagcacagccgccctgggctgcctggtgaaggactacttccccgagcccgtgaccgtgtcctggaacagcggcgctctgaccagcggcgtgcataccttccccgccgtgctccagagcagcggactgtactccctgagcagcgtggtgaccgtgccttccagcagcctgggcaccaagacctacacctgcaacgtggaccacaagcccagcaacaccaaggtggacaagagagtggagagcaagtacggccctccctgccccccttgccctgcccccgagttcgagggcggacctagcgtgttcctgttcccccccaagcccaaggacaccctgatgatcagcagaacccccgaggtgacctgcgtggtggtggacgtgtcccaggaggaccccgaggtccagtttaattggtacgtggacggcgtggaagtgcataacgccaagaccaagcccagagaggagcagttcaacagcacctacagagtggtgtccgtgctgaccgtgctgcaccaggactggctgaacggcaaggaatacaagtgcaaggtctccaacaagggcctggccagcagcatcgagaagaccatcagcaaggccaagggccagccacgggagccccaggtctacaccctgccaccttgtcaagaggagatgaccaagaaccaggtgtccctgtggtgtctggtgaaaggcttctatcccagcgatatcgccgtggagtgggagagcaacggccagcccgagaacaactacaagaccaccccccctgtgctggacagcgacggcagcttcttcctgtactccaagctgaccgtggacaagtccagatggcaggagggcaacgtcttcagctgctccgtgatgcacgaggccctgcacaaccactacacccagaagtccctgagcctgagcctgggcaag

SEQ ID NO: 110 - protein, 214 aa, Homo sapiens
EIVLTQSPGTLSLSPGERATLSCRASQSVSSYLAWYQKKPGQAPRLLIYDASNRATGIPDRFSGSGSGTDFTLTISRLEPEDFAVYYCQQRSNWPITFGQGTKLEIKRTVAAPSVFIFPPSDEQLKSGTASVVCLLNNFYPREAKVQWKVDNALQSGNSQESVTEQDSKDSTYSLSSTLTLSKADYEKHKVYACEVTHQGLSSPVTKSFNRGEC

SEQ ID NO: 111 - DNA, 642 bp, Homo sapiens
gagatcgtgctgacacagagccctggcacactgtcactgtctccaggcgagagagccacactgagctgtagagccagccagagcgtgtcctcttacctggcctggtatcagaagaagcctggacaggctcccagactgctgatctacgacgccagcaacagagccacaggcatccccgatagattcagcggctctggctctggcaccgacttcaccctgacaatcagcagactggaacccgaggacttcgccgtgtactactgccagcagagaagcaactggcccatcacattcggccagggcaccaagctggaaatcaagcgaactgtggctgcaccatctgtcttcatcttcccgccatctgatgagcagttgaaatctggaactgcctctgttgtgtgcctgctgaataacttctatcccagagaggccaaagtacagtggaaggtggataacgccctccaatcgggtaactcccaggagagtgtcacagagcaggacagcaaggacagcacctacagcctcagcagcaccctgacgctgagcaaagcagactacgagaaacacaaagtctacgcctgcgaagtcacccatcagggcctgagctcgcccgtcacaaagagcttcaacaggggagagtgt

SEQ ID NO: 112 - protein, 449 aa, Homo sapiens
EVQLLESGGGVVQPGGSLRLSCAASGFTFNDYAMHWVREAPGKGLEWVSTISWNSGSIGYADSVKGRFTISRDNSKNTLYLQMNSLRAEDTAVYYCAKDIQYGNYYYGMDYWGQGTLVTVSSASTKGPSVFPLAPCSRSTSESTAALGCLVKDYFPEPVTVSWNSGALTSGVHTFPAVLQSSGLYSLSSVVTVPSSSLGTKTYTCNVDHKPSNTKVDKRVESKYGPPCPPCPAPEFEGGPSVFLFPPKPKDTLMISRTPEVTCVVVDVSQEDPEVQFNWYVDGVEVHNAKTKPREEQFNSTYRVVSVLTVLHQDWLNGKEYKCKVSNKGLASSIEKTISKAKGQPREPQVCTLPPSQEEMTKNQVSLSCAVKGFYPSDIAVEWESNGQPENNYKTTPPVLDSDGSFFLVSKLTVDKSRWQEGNVFSCSVMHEALHNHYTQKSLSLSLGK

SEQ ID NO: 113 - DNA, 1347 bp, Homo sapiens
gaagtgcagctgctggaatctggtggcggagttgttcagcctggcggctctctgagactgtcttgtgctgccagcggcttcaccttcaacgactacgctatgcactgggtccgagaggcccctggcaaaggacttgaatgggtgtccaccatcagctggaacagcggctctatcggctacgccgattccgtgaagggcagattcaccatctccagagacaacagcaagaacaccctgtacctgcagatgaacagcctgagagccgaggacaccgccgtgtactactgtgccaaggacatccagtacggcaactactactacggcatggactactggggccagggaacactggttaccgttagctctgctagcaccaagggccccagcgtgttccccctggccccttgcagcagaagcaccagcgagagcacagccgccctgggctgcctggtgaaggactacttccccgagcccgtgaccgtgtcctggaacagcggcgctctgaccagcggcgtgcataccttccccgccgtgctccagagcagcggactgtactccctgagcagcgtggtgaccgtgccttccagcagcctgggcaccaagacctacacctgcaacgtggaccacaagcccagcaacaccaaggtggacaagagagtggagagcaagtacggccctccctgccccccttgccctgcccccgagttcgagggcggacctagcgtgttcctgttcccccccaagcccaaggacaccctgatgatcagcagaacccccgaggtgacctgcgtggtggtggacgtgtcccaggaggaccccgaggtccagtttaattggtacgtggacggcgtggaagtgcataacgccaagaccaagcccagagaggagcagttcaacagcacctacagagtggtgtccgtgctgaccgtgctgcaccaggactggctgaacggcaaggaatacaagtgcaaggtctccaacaagggcctggccagcagcatcgagaagaccatcagcaaggccaagggccagccacgggagccccaggtctgcaccctgccacctagccaagaggagatgaccaagaaccaggtgtccctgagctgtgccgtgaaaggcttctatcccagcgatatcgccgtggagtgggagagcaacggccagcccgagaacaactacaagaccaccccccctgtgctggacagcgacggcagcttcttcctggtttccaagctgaccgtggacaagtccagatggcaggagggcaacgtcttcagctgctccgtgatgcacgaggccctgcacaaccactacacccagaagtccctgagcctgagcctgggcaag

SEQ ID NO: 114 - protein, 215 aa, Homo sapiens
QAVVTQEPSLTVSPGGTVTLTCRSSTGAVTTSNYANWVQEKPGQAPRGLIGGTNKRAPWTPARFSGSLLGGKAALTITGAQAEDEAEYYCVLWYSNLWVFGGGTKLTVLGQPKAAPSVTLFPPSSEELQANKATLVCLISDFYPGAVTVAWKADSSPVKAGVETTTPSKQSNNKYAASSYLSLTPEQWKSHRSYSCQVTHEGSTVEKTVAPTECS

SEQ ID NO: 115 - DNA, 645 bp, Homo sapiens
caggctgtggtcacacaagagcctagcctgacagtgtctcctggcggcacagtgaccctgacctgtagatcttctacaggcgccgtgaccaccagcaactacgctaattgggtgcaggagaagcccggccaggctcctagaggactgatcggcggaacaaacaagagagccccttggacacccgccagattctctggatctctgctcggcggaaaggccgctctgacaatcactggtgctcaggctgaggacgaggccgagtactattgtgtgctgtggtacagcaacctgtgggtgttcggcggaggcaccaaactgacagttctgggtcagcccaaggcggcgccctcggtcactctgttcccgccctcctctgaggagcttcaagccaacaaggccacactggtgtgtctcataagtgacttctatccgggagccgtgacagtggcctggaaggcagatagcagccccgtcaaggcgggagtggagaccaccacaccctccaaacaaagcaacaacaagtacgcggccagcagctacctgagcctgacgcctgagcagtggaagtcccacagaagctacagctgccaggtcacgcatgaagggagcaccgtggagaagacagtggcccctacagaatgttca

SEQ ID NO: 116 - protein, 452 aa, Homo sapiens
EVQLVESGGGLVQPGGSLRLSCAASGFTFNTYAMNWVRKAPGKGLEWVGRIRSKYNNYATYYADSVKDRFTISRDDSKNSLYLQMNSLKTEDTAVYYCVRHGNFGNSYVSWFAYWGQGTLVTVSSASTKGPSVFPLAPCSRSTSESTAALGCLVKDYFPEPVTVSWNSGALTSGVHTFPAVLQSSGLYSLSSVVTVPSSSLGTKTYTCNVDHKPSNTKVDKRVESKYGPPCPPCPAPEFEGGPSVFLFPPKPKDTLMISRTPEVTCVVVDVSQEDPEVQFNWYVDGVEVHNAKTKPREEQFNSTYRVVSVLTVLHQDWLNGKEYKCKVSNKGLASSIEKTISKAKGQPREPQVYTLPPCQEEMTKNQVSLWCLVKGFYPSDIAVEWESNGQPENNYKTTPPVLDSDGSFFLYSKLTVDKSRWQEGNVFSCSVMHEALHNHYTQKSLSLSLGK

SEQ ID NO: 117 - DNA, 1356 bp, Homo sapiens
gaggtgcagctggttgaatctggcggaggactggttcagcctggcggatctctgagactgtcttgtgccgccagcggcttcaccttcaacacctacgctatgaactgggtccgaaaggcccctggcaaaggactggaatgggtgggaagaatcaggtccaagtacaacaactacgccacctactacgccgacagcgtgaaggacagattcaccatcagcagggacgacagcaagaacagcctgtacctgcagatgaacagcctgaaaaccgaggacaccgccgtgtactactgtgtcagacacggcaacttcggcaacagctatgtgtcttggtttgcctactggggccagggcacactggtcacagttagctctgctagcaccaagggccccagcgtgttccccctggccccttgcagcagaagcaccagcgagagcacagccgccctgggctgcctggtgaaggactacttccccgagcccgtgaccgtgtcctggaacagcggcgctctgaccagcggcgtgcataccttccccgccgtgctccagagcagcggactgtactccctgagcagcgtggtgaccgtgccttccagcagcctgggcaccaagacctacacctgcaacgtggaccacaagcccagcaacaccaaggtggacaagagagtggagagcaagtacggccctccctgccccccttgccctgcccccgagttcgagggcggacctagcgtgttcctgttcccccccaagcccaaggacaccctgatgatcagcagaacccccgaggtgacctgcgtggtggtggacgtgtcccaggaggaccccgaggtccagtttaattggtacgtggacggcgtggaagtgcataacgccaagaccaagcccagagaggagcagttcaacagcacctacagagtggtgtccgtgctgaccgtgctgcaccaggactggctgaacggcaaggaatacaagtgcaaggtctccaacaagggcctggccagcagcatcgagaagaccatcagcaaggccaagggccagccacgggagccccaggtctacaccctgccaccttgtcaagaggagatgaccaagaaccaggtgtccctgtggtgtctggtgaaaggcttctatcccagcgatatcgccgtggagtgggagagcaacggccagcccgagaacaactacaagaccaccccccctgtgctggacagcgacggcagcttcttcctgtactccaagctgaccgtggacaagtccagatggcaggagggcaacgtcttcagctgctccgtgatgcacgaggccctgcacaaccactacacccagaagtccctgagcctgagcctgggcaag

SEQ ID NO: 118 - protein, 214 aa, Homo sapiens; identical to SEQ ID NO: 96

SEQ ID NO: 119 - DNA, 642 bp, Homo sapiens; identical to SEQ ID NO: 97

SEQ ID NO: 120 - protein, 449 aa, Homo sapiens
EVQLLESGGGVVQPGGSLRLSCAASGFTFNDYAMHWVREAPGKGLEWVSTISWNSGSIGYADSVKGRFTISRDNSKNTLYLQMNSLRAEDTAVYYCAKDIQYGNYYYGMDYWGQGTLVTVSSASTKGPSVFPLAPCSRSTSESTAALGCLVEDYFPEPVTVSWNSGALTSGVHTFPAVLQSSGLYSLSSVVTVPSSSLGTKTYTCNVDHKPSNTKVDERVESKYGPPCPPCPAPEFEGGPSVFLFPPKPKDTLMISRTPEVTCVVVDVSQEDPEVQFNWYVDGVEVHNAKTKPREEQFNSTYRVVSVLTVLHQDWLNGKEYKCKVSNKGLASSIEKTISKAKGQPREPQVCTLPPSQEEMTKNQVSLSCAVKGFYPSDIAVEWESNGQPENNYKTTPPVLDSDGSFFLVSKLTVDKSRWQEGNVFSCSVMHEALHNHYTQKSLSLSLGK

SEQ ID NO: 121 - DNA, 1347 bp, Homo sapiens
gaagtgcagctgctggaatctggtggcggagttgttcagcctggcggctctctgagactgtcttgtgctgccagcggcttcaccttcaacgactacgctatgcactgggtccgagaggcccctggcaaaggacttgaatgggtgtccaccatcagctggaacagcggctctatcggctacgccgattccgtgaagggcagattcaccatctccagagacaacagcaagaacaccctgtacctgcagatgaacagcctgagagccgaggacaccgccgtgtactactgtgccaaggacatccagtacggcaactactactacggcatggactactggggccagggaacactggttaccgttagctctgctagcaccaagggccccagcgtgttccccctggccccttgcagcagaagcaccagcgagagcacagccgccctgggctgcctggtggaggactacttccccgagcccgtgaccgtgtcctggaacagcggcgctctgaccagcggcgtgcataccttccccgccgtgctccagagcagcggactgtactccctgagcagcgtggtgaccgtgccttccagcagcctgggcaccaagacctacacctgcaacgtggaccacaagcccagcaacaccaaggtggacgagagagtggagagcaagtacggccctccctgccccccttgccctgcccccgagttcgaaggcggacctagcgtgttcctgttcccccccaagcccaaggacaccctgatgatcagcagaacccccgaggtgacctgcgtggtggtggacgtgtcccaggaggaccccgaggtccagtttaattggtacgtggacggcgtggaagtgcataacgccaagaccaagcccagagaggagcagttcaacagcacctacagagtggtgtccgtgctgaccgtgctgcaccaggactggctgaacggcaaggaatacaagtgcaaggtctccaacaagggcctggccagcagcatcgagaagaccatcagcaaggccaagggccagccacgggagccccaggtctgcaccctgccacctagccaagaggagatgaccaagaaccaggtgtccctgagctgtgccgtgaaaggcttctatcccagcgatatcgccgtggagtgggagagcaacggccagcccgagaacaactacaagaccaccccccctgtgctggacagcgacggcagcttcttcctggtttccaagctgaccgtggacaagtccagatggcaggagggcaacgtcttcagctgctccgtgatgcacgaggccctgcacaaccactacacccagaagtccctgagcctgagcctgggcaag

SEQ ID NO: 122 - protein, 109 aa, Mus musculus
QAVVTQESALTTSPGETVTLTCRSSTGAVTTSNYANWVQQKPDHLFTGLIGGTNKRAPGVPARFSGSLIGDKAALTITGAQTEDEAIYFCALWYSNLWVFGGGTKLTVL

SEQ ID NO: 123 - protein, 125 aa, Mus musculus
EVQLVESGGGLVQPKGSLKLSCAASGFTFNTYAMNWVRQAPGKGLEWVARIRSKYNNYATYYADSVKDRFTISRDDSQSILYLQMNNLKTEDTAMYYCVRHGNFGNSYVSWFAYWGQGTLVTVSS